European Patent Application EP 4 215 544 A1, published July 26, 2023. Title: MONOCLONAL ANTIBODY FOR CORONAVIRUS SPIKE PROTEIN, AND USE THEREOF. Applicant: Innovent Biologics (Suzhou) Co., Ltd. The sequence listing filed with the application follows.

SEQUENCE LISTING (70 sequences)

SEQ ID NO: 1 - DNA, 360 bp, Artificial sequence
  VH of antibody P5-22
gaggtgcagctggtggagtctgggggaggcttggtcaagcctggagggtccctgagactctcctgtgcagcctctggattcaccttcagggactacgacatcatctggatccgccaggctccagggaaggggctggagtgggtttcatacattagtcgtagtggtagtaccatatactactcagactctgtgaggggccgattcaccatctccagggacaacgccaagaattcagtgtatctgcaaatgaacagcctgagagccgaggacacggccgtgtattactgtgcgagagatttcgggtttgagggaccccgtatggacgtctggggccaagggaccacggtcaccgtctcctca

SEQ ID NO: 2 - protein, 120 aa, Artificial sequence
  VH of antibody P5-22
EVQLVESGGGLVKPGGSLRLSCAASGFTFRDYDIIWIRQAPGKGLEWVSYISRSGSTIYYSDSVRGRFTISRDNAKNSVYLQMNSLRAEDTAVYYCARDFGFEGPRMDVWGQGTTVTVSS

SEQ ID NO: 3 - DNA, 321 bp, Artificial sequence
  VL of antibody P5-22
gacatccagatgacccagtctccatcctccctgtctgcatctgtaggagacagagtcaccatcacttgccaggcgagtcaggacattaagaactatttaaattggtatcagcagaaaccagggaaagcccctaagctcctgatctacgatgcatccaatttggaaacaggggtcccatcaaggttcagtggaagtggatctgggacagattttactttcaccatcagcagcctgcagcctgaagatattgcaacatattactgtcaacagtttgataatctcccgatcaccttcggccaagggacacgactggagattaaa

SEQ ID NO: 4 - protein, 107 aa, Artificial sequence
  VL of antibody P5-22
DIQMTQSPSSLSASVGDRVTITCQASQDIKNYLNWYQQKPGKAPKLLIYDASNLETGVPSRFSGSGSGTDFTFTISSLQPEDIATYYCQQFDNLPITFGQGTRLEIK

SEQ ID NO: 5 - DNA, 384 bp, Artificial sequence
  VH of antibody P14-44
caggtgcagctggtgcagtctggggctgaggtgaagaagcctggggcctcagtgaaggtttcctgcaaggcatctggatacattttcaccagctattctatgcactgggtgcgacaggcccctggacaagggcttgagtggatgggaacaatcaagcctagtgatgatagcacaaactacgcacagaagttccagggcagagtctccatgaccagggacacgtccacgagcacagtctacatggagctgagcagcctgagatatgaggacacggccgtgtattactgtgcgagagaggcccggggatattatgatagaagtggttattaccacccgggttactttgactactggggccagggaaccctggtcaccgtctcctca

SEQ ID NO: 6 - protein, 128 aa, Artificial sequence
  VH of antibody P14-44
QVQLVQSGAEVKKPGASVKVSCKASGYIFTSYSMHWVRQAPGQGLEWMGTIKPSDDSTNYAQKFQGRVSMTRDTSTSTVYMELSSLRYEDTAVYYCAREARGYYDRSGYYHPGYFDYWGQGTLVTVSS

SEQ ID NO: 7 - DNA, 330 bp, Artificial sequence
  VL of antibody P14-44
cagtctgtgctgactcagcctgcctccgtgtctgggtctcctggacagtcgatcaccatctcctgcactggaaccagcagtgacgttggtggttataactttgtctcctggtaccaacagcacccaggcaaagcccccaaactcatgatttatgaggtcagtgatcggccctcaggggtttctagtcgcttctctggctccaagtctggcaacacggcctccctgaccatctctgggctccaggctgaggacgaggctgattattactgcttctcatatacaaccagcaccacttgggtgttcggcggagggaccaagctgaccgtccta

SEQ ID NO: 8 - protein, 110 aa, Artificial sequence
  VL of antibody P14-44
QSVLTQPASVSGSPGQSITISCTGTSSDVGGYNFVSWYQQHPGKAPKLMIYEVSDRPSGVSSRFSGSKSGNTASLTISGLQAEDEADYYCFSYTTSTTWVFGGGTKLTVL

SEQ ID NO: 9 - DNA, 384 bp, Artificial sequence
  VH of antibody P15-16
caggtgcagctggtggagtctgggggaggcttggtacagcctggcaggtccctgacactctcctgtgcagcctctggattcacctttgatgattatgccatgcactgggtccggcaagctccagggaagggcctggagtgggtctcaggtattagttggaatagtggtaccatagactatgcggactctgtgaagggccgattcaccatctccagagacaacgccaagaactccctgtatctgcaaatgaacagtctgagagctgaggacacggccttgtattactgtgcaaccctcccacgtgaacgtgcatatagtggctacgatcgaatcttctacactatagacgtctggggccaagggaccacggtcaccgtctcctca

SEQ ID NO: 10 - protein, 128 aa, Artificial sequence
  VH of antibody P15-16
QVQLVESGGGLVQPGRSLTLSCAASGFTFDDYAMHWVRQAPGKGLEWVSGISWNSGTIDYADSVKGRFTISRDNAKNSLYLQMNSLRAEDTALYYCATLPRERAYSGYDRIFYTIDVWGQGTTVTVSS

SEQ ID NO: 11 - DNA, 321 bp, Artificial sequence
  VL of antibody P15-16
gacatccagatgacccagtctccatcctccctgtctgcatctgtaggagacagagtcaccatcacttgccgggcaagtcagagcattagcacctatttaaattggtatcagcagaaaccagggaaagcccctaagctcctgatctatgctgcatccagtttgcaaagtggggtcccatcaaggttcagtggcagtggatctgggacagatttcactctcaccatcagcagtctgcaacctgaagattttgcaacctactactgtcaacagagttacagtacccctctcactttcggcggagggaccaaggtggaaatcaaa

SEQ ID NO: 12 - protein, 107 aa, Artificial sequence
  VL of antibody P15-16
DIQMTQSPSSLSASVGDRVTITCRASQSISTYLNWYQQKPGKAPKLLIYAASSLQSGVPSRFSGSGSGTDFTLTISSLQPEDFATYYCQQSYSTPLTFGGGTKVEIK

SEQ ID NO: 13 - DNA, 369 bp, Artificial sequence
  VH of antibody P10-20
caggtgcagctggtggagtctgggggaggcttggtcaagcctggagggtccctgagactctcctgtgcagcctctggattcaccttcagtgactactacatgagctggatccgccaggctccagggaaggggctggagtgggtttcatacattagtattagtagtacttacacaaactacgcagactctgtgaagggccgattcaccatctccagagacaacgccaagaactcactgtatctgcaaatgaacagcctgagagccgaggacacggccgtgtattactgtgtgatagcagcagctggtaagggtcactactactacggtatggacgtctggggccaagggaccacggtcaccgtctcctca

SEQ ID NO: 14 - protein, 123 aa, Artificial sequence
  VH of antibody P10-20
QVQLVESGGGLVKPGGSLRLSCAASGFTFSDYYMSWIRQAPGKGLEWVSYISISSTYTNYADSVKGRFTISRDNAKNSLYLQMNSLRAEDTAVYYCVIAAAGKGHYYYGMDVWGQGTTVTVSS

SEQ ID NO: 15 - DNA, 321 bp, Artificial sequence
  VL of antibody P10-20
gacatccagatgacccagtctccatcctccctgtctgcatctgtaggagacagagtcaccatcacttgccaggcgagtcaggacattagcaactatttaaattggtatcagcagaaaccagggaaagcccctaagctcctgatctacgatgcatccagtttggaaacaggggtcccatcaaggttcagtggaagtggatctgggacagattttactttcaccatcagcagcctgcagcctgaagatattgcaacatattactgtcaacagtatgataatctcccgctcactttcggcggagggaccaaggtggagatcaaa

SEQ ID NO: 16 - protein, 107 aa, Artificial sequence
  VL of antibody P10-20
DIQMTQSPSSLSASVGDRVTITCQASQDISNYLNWYQQKPGKAPKLLIYDASSLETGVPSRFSGSGSGTDFTFTISSLQPEDIATYYCQQYDNLPLTFGGGTKVEIK

SEQ ID NO: 17 - DNA, 390 bp, Artificial sequence
  VH of antibody P14-37
gaggtgcagctggtggagtctgggggaggcttggtaaagcctggggggtcccttagactctcctgtgccgcctctggattcactttcagtaacgcctggatgagctgggtccgccaggctccagggaagggcctggagtgggttggccgtattaaaaggaatagcgatggtgggacaacagaccacgctgcacccgtgacaggcagattcatcatctcaagagatgattcaaaaaacacgctgtatctgcaaatgaacagcctgagaaccgaggacacagccgtctattactgtaccacagatctggatactgtagttcggcgagttgttataaccgatcatgatgcttttgatatctggggccaagggacaatggtcaccgtctcttca

SEQ ID NO: 18 - protein, 130 aa, Artificial sequence
  VH of antibody P14-37
EVQLVESGGGLVKPGGSLRLSCAASGFTFSNAWMSWVRQAPGKGLEWVGRIKRNSDGGTTDHAAPVTGRFIISRDDSKNTLYLQMNSLRTEDTAVYYCTTDLDTVVRRVVITDHDAFDIWGQGTMVTVSS

SEQ ID NO: 19 - DNA, 324 bp, Artificial sequence
  VL of antibody P14-37
gacatccagatgacccagtctccatcctccctatctgcatctgtaggagacagagtcaccatcacttgccgggcaagtcagagcattagcagctttttaaattggtatcagcagaaagcagggaaagcccctaagctcctgatctatgctgcatccagtttgcaaagtggggtcccatcaaggttcagtggcagtggatctgggacagatttcagtctcaccatcagcaatctgcaacctgaagattttgcaacttactactgtcaacagagttacagtaccccttcgatcaccttcggccaagggacacgactggagattaaa

SEQ ID NO: 20 - protein, 108 aa, Artificial sequence
  VL of antibody P14-37
DIQMTQSPSSLSASVGDRVTITCRASQSISSFLNWYQQKAGKAPKLLIYAASSLQSGVPSRFSGSGSGTDFSLTISNLQPEDFATYYCQQSYSTPSITFGQGTRLEIK

SEQ ID NO: 21 - DNA, 351 bp, Artificial sequence
  VH of antibody P23-29
caggtgcagctgcaggagtcgggcccaggactggtgaagccttcggagaccctgtccctcacctgcactgtctctggtgactccatcagcagtagtacttactactggggctggatccgccagcccccagggaaggggctggagtggattgggagtatgtattatggtcggagtacctactacaacccgtccctcaagagtcgagtcaccgtatccgtagacacgtccaagaaccagttgtccctgaaggtgagctctgtgaccgccgcagacacggctgtctattactgtgcgagacatctgggtggcgttgactactggggccagggaaccctggtcaccgtctcttca

SEQ ID NO: 22 - protein, 117 aa, Artificial sequence
  VH of antibody P23-29
QVQLQESGPGLVKPSETLSLTCTVSGDSISSSTYYWGWIRQPPGKGLEWIGSMYYGRSTYYNPSLKSRVTVSVDTSKNQLSLKVSSVTAADTAVYYCARHLGGVDYWGQGTLVTVSS

SEQ ID NO: 23 - DNA, 324 bp, Artificial sequence
  VL of antibody P23-29
gacatccagatgacccagtctccatcctccctgtctgcatctgtaggagacagagtcaccatcacttgccgggcgagtcagggcattagcaattctttagcctggtatcagcaggaaccagggaaagcccctaagctcctgctctatgctgcatccacattggaaagtggggtcccatccaggttcagtggcagtgggtctggggcggattccactctcaccatcagcagcctgcagcctgaagattttgcaacttattactgtcaacagtattatagtgcctccgcgctcactttcggcggagggaccaaggtggagattaaa

SEQ ID NO: 24 - protein, 108 aa, Artificial sequence
  VL of antibody P23-29
DIQMTQSPSSLSASVGDRVTITCRASQGISNSLAWYQQEPGKAPKLLLYAASTLESGVPSRFSGSGSGADSTLTISSLQPEDFATYYCQQYYSASALTFGGGTKVEIK

SEQ ID NO: 25 - DNA, 354 bp, Artificial sequence
  VH of antibody P3-11
caggtgcagctggtggagtctgggggaggcttggtccagcctggggggtccctgagactctcctgtgcagcctctggaatcaccgtcagtagcaactatatgagctgggtccgccaggctccagggaaggggctggaatgggtctcagttatttatagcggtggtagcacattctacgcagaccccgtgaagggcagactcaccatctccagagacaattccaagaacacgctgtatcttcaaatgaacagtgtgagagtcgaggacacggctgtgtattactgtgcgagaggagaaggatgggagctgccatttgactactggggccagggagccctggtcaccgtctcctca

SEQ ID NO: 26 - protein, 118 aa, Artificial sequence
  VH of antibody P3-11
QVQLVESGGGLVQPGGSLRLSCAASGITVSSNYMSWVRQAPGKGLEWVSVIYSGGSTFYADPVKGRLTISRDNSKNTLYLQMNSVRVEDTAVYYCARGEGWELPFDYWGQGALVTVSS

SEQ ID NO: 27 - DNA, 330 bp, Artificial sequence
  VL of antibody P3-11
cagtctgagctgactcagcctccctccgcgtccgggtctcctggacagtcagtcaccatctcctgcactggaaccagcagtgacgttggtggtaataaatatgtctcctggtaccaacagcacccaggcaaagcccccaaactcataatttatgaggtcagtaagcggccctcaggggtccctgatcgcttctctggctccaagtctggcaacacggcctccctgaccgtctctgggctccaggctgaggatgaggctgattatcactgcagctcatatgcaggcagcaacaatttggtgttcggcggagggaccaagctgaccgtccta

SEQ ID NO: 28 - protein, 110 aa, Artificial sequence
  VL of antibody P3-11
QSALTQPPSASGSPGQSVTISCTGTSSDVGGNKYVSWYQQHPGKAPKLIIYEVSKRPSGVPDRFSGSKSGNTASLTVSGLQAEDEADYHCSSYAGSNNLVFGGGTKLTVL

SEQ ID NO: 29 - protein, 10 aa, Artificial sequence
  HCDR1 of antibody P5-22 (AbM numbering)
GFTFRDYDII

SEQ ID NO: 30 - protein, 17 aa, Artificial sequence
  HCDR2 of antibody P5-22 (Kabat numbering)
YISRSGSTIYYSDSVRG

SEQ ID NO: 31 - protein, 11 aa, Artificial sequence
  HCDR3 of antibody P5-22 (Kabat numbering)
DFGFEGPRMDV

SEQ ID NO: 32 - protein, 11 aa, Artificial sequence
  LCDR1 of antibody P5-22 (Kabat numbering)
QASQDIKNYLN

SEQ ID NO: 33 - protein, 7 aa, Artificial sequence
  LCDR2 of antibody P5-22 (Kabat numbering)
DASNLET

SEQ ID NO: 34 - protein, 9 aa, Artificial sequence
  LCDR3 of antibody P5-22 (Kabat numbering)
QQFDNLPIT

SEQ ID NO: 35 - protein, 10 aa, Artificial sequence
  HCDR1 of antibody P14-44 (AbM numbering)
GYIFTSYSMH

SEQ ID NO: 36 - protein, 17 aa, Artificial sequence
  HCDR2 of antibody P14-44 (Kabat numbering)
TIKPSDDSTNYAQKFQG

SEQ ID NO: 37 - protein, 19 aa, Artificial sequence
  HCDR3 of antibody P14-44 (Kabat numbering)
EARGYYDRSGYYHPGYFDY

SEQ ID NO: 38 - protein, 14 aa, Artificial sequence
  LCDR1 of antibody P14-44 (Kabat numbering)
TGTSSDVGGYNFVS

SEQ ID NO: 39 - protein, 7 aa, Artificial sequence
  LCDR2 of antibody P14-44 (Kabat numbering)
EVSDRPS

SEQ ID NO: 40 - protein, 10 aa, Artificial sequence
  LCDR3 of antibody P14-44 (Kabat numbering)
FSYTTSTTWV

SEQ ID NO: 41 - protein, 10 aa, Artificial sequence
  HCDR1 of antibody P15-16 (AbM numbering)
GFTFDDYAMH

SEQ ID NO: 42 - protein, 17 aa, Artificial sequence
  HCDR2 of antibody P15-16 (Kabat numbering)
GISWNSGTIDYADSVKG

SEQ ID NO: 43 - protein, 19 aa, Artificial sequence
  HCDR3 of antibody P15-16 (Kabat numbering)
LPRERAYSGYDRIFYTIDV

SEQ ID NO: 44 - protein, 11 aa, Artificial sequence
  LCDR1 of antibody P15-16 (Kabat numbering)
RASQSISTYLN

SEQ ID NO: 45 - protein, 7 aa, Artificial sequence
  LCDR2 of antibody P15-16 (Kabat numbering)
AASSLQS

SEQ ID NO: 46 - protein, 9 aa, Artificial sequence
  LCDR3 of antibody P15-16 (Kabat numbering)
QQSYSTPLT

SEQ ID NO: 47 - protein, 10 aa, Artificial sequence
  HCDR1 of antibody P10-20 (AbM numbering)
GFTFSDYYMS

SEQ ID NO: 48 - protein, 17 aa, Artificial sequence
  HCDR2 of antibody P10-20 (Kabat numbering)
YISISSTYTNYADSVKG

SEQ ID NO: 49 - protein, 14 aa, Artificial sequence
  HCDR3 of antibody P10-20 (Kabat numbering)
AAAGKGHYYYGMDV

SEQ ID NO: 50 - protein, 11 aa, Artificial sequence
  LCDR1 of antibody P10-20 (Kabat numbering)
QASQDISNYLN

SEQ ID NO: 51 - protein, 7 aa, Artificial sequence
  LCDR2 of antibody P10-20 (Kabat numbering)
DASSLET

SEQ ID NO: 52 - protein, 9 aa, Artificial sequence
  LCDR3 of antibody P10-20 (Kabat numbering)
QQYDNLPLT

SEQ ID NO: 53 - protein, 10 aa, Artificial sequence
  HCDR1 of antibody P14-37 (AbM numbering)
GFTFSNAWMS

SEQ ID NO: 54 - protein, 19 aa, Artificial sequence
  HCDR2 of antibody P14-37 (Kabat numbering)
RIKRNSDGGTTDHAAPVTG

SEQ ID NO: 55 - protein, 19 aa, Artificial sequence
  HCDR3 of antibody P14-37 (Kabat numbering)
DLDTVVRRVVITDHDAFDI

SEQ ID NO: 56 - protein, 11 aa, Artificial sequence
  LCDR1 of antibody P14-37 (Kabat numbering)
RASQSISSFLN

SEQ ID NO: 57 - protein, 7 aa, Artificial sequence
  LCDR2 of antibody P14-37 (Kabat numbering)
AASSLQS

SEQ ID NO: 58 - protein, 10 aa, Artificial sequence
  LCDR3 of antibody P14-37 (Kabat numbering)
QQSYSTPSIT

SEQ ID NO: 59 - protein, 12 aa, Artificial sequence
  HCDR1 of antibody P23-29 (AbM numbering)
GDSISSSTYYWG

SEQ ID NO: 60 - protein, 16 aa, Artificial sequence
  HCDR2 of antibody P23-29 (Kabat numbering)
SMYYGRSTYYNPSLKS

SEQ ID NO: 61 - protein, 7 aa, Artificial sequence
  HCDR3 of antibody P23-29 (Kabat numbering)
HLGGVDY

SEQ ID NO: 62 - protein, 11 aa, Artificial sequence
  LCDR1 of antibody P23-29 (Kabat numbering)
RASQGISNSLA

SEQ ID NO: 63 - protein, 7 aa, Artificial sequence
  LCDR2 of antibody P23-29 (Kabat numbering)
AASTLES

SEQ ID NO: 64 - protein, 10 aa, Artificial sequence
  LCDR3 of antibody P23-29 (Kabat numbering)
QQYYSASALT

SEQ ID NO: 65 - protein, 10 aa, Artificial sequence
  HCDR1 of antibody P3-11 (AbM numbering)
GITVSSNYMS

SEQ ID NO: 66 - protein, 16 aa, Artificial sequence
  HCDR2 of antibody P3-11 (Kabat numbering)
VIYSGGSTFYADPVKG

SEQ ID NO: 67 - protein, 10 aa, Artificial sequence
  HCDR3 of antibody P3-11 (Kabat numbering)
GEGWELPFDY

SEQ ID NO: 68 - protein, 14 aa, Artificial sequence
  LCDR1 of antibody P3-11 (Kabat numbering)
TGTSSDVGGNKYVS

SEQ ID NO: 69 - protein, 7 aa, Artificial sequence
  LCDR2 of antibody P3-11 (Kabat numbering)
EVSKRPS

SEQ ID NO: 70 - protein, 10 aa, Artificial sequence
  LCDR3 of antibody P3-11 (Kabat numbering)
SSYAGSNNLV